European Patent Application EP 4 296 676 A1, published December 27, 2023. Title: Method for prediction of survival rate and its use. Applicant: Mosaiques diagnostics and therapeutics AG. The sequence listing filed with the application follows.

SEQUENCE LISTING (71 sequences)

SEQ ID NO: 1 - protein, 9 aa, human
  MOD_RES (8)..(8): 4Hyp
DDGEAGKPG

SEQ ID NO: 2 - protein, 10 aa, human
  MOD_RES (7)..(7): 4Hyp
DGKTGPPGPA

SEQ ID NO: 3 - protein, 11 aa, human
  MOD_RES (4)..(4): 4Hyp
  MOD_RES (7)..(7): 4Hyp
  MOD_RES (10)..(10): 4Hyp
DGRPGPPGPPG

SEQ ID NO: 4 - protein, 12 aa, human
  MOD_RES (8)..(8): 4Hyp
  MOD_RES (11)..(11): 4Hyp
DDGEAGKPGRPG

SEQ ID NO: 5 - protein, 13 aa, human
  MOD_RES (6)..(6): 4Hyp
  MOD_RES (9)..(9): 4Hyp
  MOD_RES (11)..(11): 4Hyp
GQDGRPGPPGPPG

SEQ ID NO: 6 - protein, 15 aa, human
  MOD_RES (2)..(2): 4Hyp
PPGPAGKEGGKGPRG

SEQ ID NO: 7 - protein, 15 aa, human
  MOD_RES (3)..(3): 4Hyp
  MOD_RES (9)..(9): 4Hyp
GPPGEAGKPGEQGVP

SEQ ID NO: 8 - protein, 15 aa, human
  MOD_RES (2)..(2): 4Hyp
  MOD_RES (14)..(14): 4Hyp
PPGKNGDDGEAGKPG

SEQ ID NO: 9 - protein, 15 aa, human
  MOD_RES (2)..(2): 4Hyp
  MOD_RES (8)..(8): 4Hyp
SPGRDGSPGAKGDRG

SEQ ID NO: 10 - protein, 16 aa, human
  MOD_RES (10)..(10): 4Hyp
DGQPGAKGEPGDAGAK

SEQ ID NO: 11 - protein, 14 aa, human
  MOD_RES (8)..(8): 4Hyp
  MOD_RES (11)..(11): 4Hyp
DDGEAGKPGRPGER

SEQ ID NO: 12 - protein, 16 aa, human
  MOD_RES (4)..(4): 4Hyp
DGSPGAKGDRGETGPA

SEQ ID NO: 13 - protein, 17 aa, human
  MOD_RES (3)..(3): 4Hyp
  MOD_RES (9)..(9): 4Hyp
VGPPGPPGPPGPPGPPS

SEQ ID NO: 14 - protein, 16 aa, human
  MOD_RES (3)..(3): 4Hyp
  MOD_RES (9)..(9): 4Hyp
GSPGRDGSPGAKGDRG

SEQ ID NO: 15 - protein, 17 aa, human
  MOD_RES (4)..(4): 4Hyp
  MOD_RES (10)..(10): 4Hyp
  MOD_RES (13)..(13): 4Hyp
VGPPGPPGPPGPPGPPS

SEQ ID NO: 16 - protein, 18 aa, human
  MOD_RES (4)..(4): 4Hyp
  MOD_RES (7)..(7): 4Hyp
  MOD_RES (13)..(13): 4Hyp
VGPPGPPGPPGPPGPPSA

SEQ ID NO: 17 - protein, 20 aa, human
  MOD_RES (4)..(4): 4Hyp
  MOD_RES (16)..(16): 4Hyp
  MOD_RES (19)..(19): 4Hyp
NGAPGNDGAKGDAGAPGAPG

SEQ ID NO: 18 - protein, 19 aa, human
  MOD_RES (2)..(2): 4Hyp
  MOD_RES (5)..(5): 4Hyp
  MOD_RES (18)..(18): 4Hyp
GPPGPPGKNGDDGEAGKPG

SEQ ID NO: 19 - protein, 19 aa, human
  MOD_RES (4)..(4): 4Hyp
  MOD_RES (10)..(10): 4Hyp
EGSPGRDGSPGAKGDRGET

SEQ ID NO: 20 - protein, 21 aa, human
  MOD_RES (11)..(11): 4Hyp
  MOD_RES (14)..(14): 4Hyp
  MOD_RES (20)..(20): 4Hyp
DAGPAGPKGEPGSPGENGAPG

SEQ ID NO: 21 - protein, 19 aa, human
  MOD_RES (11)..(11): 4Hyp
  MOD_RES (16)..(16): 4Hyp
DDGEAGKPGRPGERGPPGP

SEQ ID NO: 22 - protein, 19 aa, human
  MOD_RES (11)..(11): 4Hyp
  MOD_RES (16)..(16): 4Hyp
  MOD_RES (19)..(19): 4Hyp
DDGEAGKPGRPGERGPPGP

SEQ ID NO: 23 - protein, 22 aa, human
  MOD_RES (6)..(6): 4Hyp
  MOD_RES (11)..(11): 4Hyp
  MOD_RES (21)..(21): 4Hyp
GPSGEPGKQGPSGASGERGPPG

SEQ ID NO: 24 - protein, 21 aa, human
  MOD_RES (4)..(4): 4Hyp
  MOD_RES (10)..(10): 4Hyp
EGSPGRDGSPGAKGDRGETGP

SEQ ID NO: 25 - protein, 23 aa, human
  MOD_RES (7)..(7): 4Hyp
  MOD_RES (13)..(13): 4Hyp
  MOD_RES (19)..(19): 4Hyp
AGPKGSPGEAGRPGEAGLPGAKG

SEQ ID NO: 26 - protein, 22 aa, human
  MOD_RES (3)..(3): 4Hyp
  MOD_RES (6)..(6): 4Hyp
  MOD_RES (18)..(18): 4Hyp
  MOD_RES (21)..(21): 4Hyp
GPPGPPGKNGDDGEAGKPGRPG

SEQ ID NO: 27 - protein, 22 aa, human
  MOD_RES (4)..(4): 4Hyp
  MOD_RES (10)..(10): 4Hyp
EGSPGRDGSPGAKGDRGETGPA

SEQ ID NO: 28 - protein, 24 aa, human
  MOD_RES (8)..(8): 4Hyp
NSGEPGAPGSKGDTGAKGEPGPVG

SEQ ID NO: 29 - protein, 23 aa, human
  MOD_RES (5)..(5): 4Hyp
  MOD_RES (11)..(11): 4Hyp
AEGSPGRDGSPGAKGDRGETGPA

SEQ ID NO: 30 - protein, 24 aa, human
  MOD_RES (5)..(5): 4Hyp
  MOD_RES (8)..(8): 4Hyp
  MOD_RES (20)..(20): 4Hyp
  MOD_RES (24)..(24): 4Hyp
NSGEPGAPGSKGDTGAKGEPGPVG

SEQ ID NO: 31 - protein, 26 aa, human
  MOD_RES (4)..(4): 4Hyp
  MOD_RES (10)..(10): 4Hyp
IGPPGPAGAPGDKGESGPSGPAGPTG

SEQ ID NO: 32 - protein, 25 aa, human
  MOD_RES (15)..(15): 4Hyp
  MOD_RES (17)..(17): 4Hyp
  MOD_RES (18)..(18): 4Hyp
  MOD_RES (20)..(20): 4Hyp
GRTGDAGPVGPPGPPGPPGPPGPPS

SEQ ID NO: 33 - protein, 27 aa, human
  MOD_RES (5)..(5): 4Hyp
  MOD_RES (17)..(17): 4Hyp
  MOD_RES (20)..(20): 4Hyp
ANGAPGNDGAKGDAGAPGAPGSQGAPG

SEQ ID NO: 34 - protein, 26 aa, human
  MOD_RES (5)..(5): 4Hyp
  MOD_RES (11)..(11): 4Hyp
  MOD_RES (23)..(23): 4Hyp
  MOD_RES (25)..(25): 4Hyp
ADGQPGAKGEPGDAGAKGDAGPPGPA

SEQ ID NO: 35 - protein, 23 aa, human
  MOD_RES (11)..(11): 4Hyp
  MOD_RES (19)..(19): 4Hyp
  MOD_RES (20)..(20): 4Hyp
KNGDDGEAGKPGRPGERGPPGPQ

SEQ ID NO: 36 - protein, 28 aa, human
  MOD_RES (6)..(6): 4Hyp
  MOD_RES (18)..(18): 4Hyp
  MOD_RES (21)..(21): 4Hyp
  MOD_RES (27)..(27): 4Hyp
GANGAPGNDGAKGDAGAPGAPGSQGAPG

SEQ ID NO: 37 - protein, 28 aa, human
  MOD_RES (2)..(2): 4Hyp
  MOD_RES (19)..(19): 4Hyp
  MOD_RES (20)..(20): 4Hyp
APGPAGARGNDGATGAAGPPGPTGPAGP

SEQ ID NO: 38 - protein, 24 aa, human
  MOD_RES (15)..(15): 4Hyp
  MOD_RES (21)..(21): 4Hyp
  MOD_RES (23)..(23): 4Hyp
GKNGDDGEAGKPGRPGERGPPGPQ

SEQ ID NO: 39 - protein, 29 aa, human
  MOD_RES (6)..(6): 4Hyp
  MOD_RES (21)..(21): 4Hyp
TGPIGPPGPAGAPGDKGESGPSGPAGPTG

SEQ ID NO: 40 - protein, 26 aa, human
  MOD_RES (3)..(3): 4Hyp
  MOD_RES (15)..(15): 4Hyp
  MOD_RES (18)..(18): 4Hyp
GPPGKNGDDGEAGKPGRPGERGPPGP

SEQ ID NO: 41 - protein, 30 aa, human
  MOD_RES (7)..(7): 4Hyp
  MOD_RES (8)..(8): 4Hyp
LTGPIGPPGPAGAPGDKGESGPSGPAGPTG

SEQ ID NO: 42 - protein, 27 aa, human
  MOD_RES (3)..(3): 4Hyp
  MOD_RES (18)..(18): 4Hyp
  MOD_RES (24)..(24): 4Hyp
  MOD_RES (26)..(26): 4Hyp
GPPGKNGDDGEAGKPGRPGERGPPGPQ

SEQ ID NO: 43 - protein, 30 aa, human
  MOD_RES (16)..(16): 4Hyp
  MOD_RES (29)..(29): 4Hyp
KDGEAGAQGPPGPAGPAGERGEQGPAGSPG

SEQ ID NO: 44 - protein, 30 aa, human
  MOD_RES (17)..(17): 4Hyp
  MOD_RES (23)..(23): 4Hyp
  MOD_RES (26)..(26): 4Hyp
KEGGKGPRGETGPAGRPGEVGPPGPPGPAG

SEQ ID NO: 45 - protein, 28 aa, human
  MOD_RES (4)..(4): 4Hyp
  MOD_RES (7)..(7): 4Hyp
  MOD_RES (19)..(19): 4Hyp
  MOD_RES (22)..(22): 4Hyp
RGPPGPPGKNGDDGEAGKPGRPGERGPP

SEQ ID NO: 46 - protein, 32 aa, human
  MOD_RES (3)..(3): 4Hyp
  MOD_RES (9)..(9): 4Hyp
  MOD_RES (15)..(15): 4Hyp
  MOD_RES (26)..(26): 4Hyp
GPPGADGQPGAKGEPGDAGAKGDAGPPGPAGP

SEQ ID NO: 47 - protein, 31 aa, human
  MOD_RES (3)..(3): 4Hyp
  MOD_RES (12)..(12): 4Hyp
  MOD_RES (15)..(15): 4Hyp
  MOD_RES (27)..(27): 4Hyp
GPPGPKGNSGEPGAPGSKGDTGAKGEPGPVG

SEQ ID NO: 48 - protein, 32 aa, human
PGPAGPPGEAGKPGEQGVPGDLGAPGPSGARG

SEQ ID NO: 49 - protein, 30 aa, human
  MOD_RES (4)..(4): 4Hyp
  MOD_RES (7)..(7): 4Hyp
  MOD_RES (22)..(22): 4Hyp
  MOD_RES (28)..(28): 4Hyp
RGPPGPPGKNGDDGEAGKPGRPGERGPPGP

SEQ ID NO: 50 - protein, 31 aa, human
  MOD_RES (20)..(20): 4Hyp
  MOD_RES (31)..(31): 4Hyp
ESGREGAPGAEGSPGRDGSPGAKGDRGETGP

SEQ ID NO: 51 - protein, 33 aa, human
  MOD_RES (5)..(5): 4Hyp
  MOD_RES (8)..(8): 4Hyp
  MOD_RES (20)..(20): 4Hyp
  MOD_RES (29)..(29): 4Hyp
NSGEPGAPGSKGDTGAKGEPGPVGVQGPPGPAG

SEQ ID NO: 52 - protein, 33 aa, human
  MOD_RES (5)..(5): 4Hyp
  MOD_RES (8)..(8): 4Hyp
  MOD_RES (10)..(10): 4Hyp
  MOD_RES (29)..(29): 4Hyp
  MOD_RES (31)..(31): 4Hyp
  MOD_RES (32)..(32): 4Hyp
LTGSPGSPGPDGKTGPPGPAGQDGRPGPPGPPG

SEQ ID NO: 53 - protein, 32 aa, human
  MOD_RES (8)..(8): 4Hyp
  MOD_RES (20)..(20): 4Hyp
  MOD_RES (31)..(31): 4Hyp
ESGREGAPGAEGSPGRDGSPGAKGDRGETGPA

SEQ ID NO: 54 - protein, 34 aa, human
  MOD_RES (22)..(22): 4Hyp
  MOD_RES (28)..(28): 4Hyp
RGAPGDRGEPGPPGPAGFAGPPGADGQPGAKGEP

SEQ ID NO: 55 - protein, 36 aa, human
  MOD_RES (18)..(18): 4Hyp
  MOD_RES (24)..(24): 4Hyp
GPPGPAGFAGPPGADGQPGAKGEPGDAGAKGDAGPP

SEQ ID NO: 56 - protein, 34 aa, human
  MOD_RES (2)..(2): 4Hyp
  MOD_RES (11)..(11): 4Hyp
  MOD_RES (17)..(17): 4Hyp
PPGESGREGAPGAEGSPGRDGSPGAKGDRGETGP

SEQ ID NO: 57 - protein, 34 aa, human; identical to SEQ ID NO: 56
  MOD_RES (2)..(2): 4Hyp
  MOD_RES (11)..(11): 4Hyp
  MOD_RES (17)..(17): 4Hyp
  MOD_RES (23)..(23): 4Hyp

SEQ ID NO: 58 - protein, 35 aa, human
  MOD_RES (3)..(3): 4Hyp
  MOD_RES (18)..(18): 4Hyp
  MOD_RES (35)..(35): 4Hyp
GPPGESGREGAPGAEGSPGRDGSPGAKGDRGETGP

SEQ ID NO: 59 - protein, 37 aa, human
  MOD_RES (5)..(5): 4Hyp
  MOD_RES (14)..(14): 4Hyp
  MOD_RES (17)..(17): 4Hyp
AAGEPGKAGERGVPGPPGAVGPAGKDGEAGAQGPPGP

SEQ ID NO: 60 - protein, 35 aa, human; identical to SEQ ID NO: 58
  MOD_RES (3)..(3): 4Hyp
  MOD_RES (18)..(18): 4Hyp
  24MOD_RES (24)..(24): 4Hyp
  24MOD_RES (35)..(35): 4Hyp

SEQ ID NO: 61 - protein, 37 aa, human
  MOD_RES (28)..(28): 4Hyp
  MOD_RES (30)..(30): 4Hyp
KGESGPSGPAGPTGARGAPGDRGEPGPPGPAGFAGPP

SEQ ID NO: 62 - protein, 38 aa, human
  MOD_RES (4)..(4): 4Hyp
  MOD_RES (10)..(10): 4Hyp
  MOD_RES (13)..(13): 4Hyp
  MOD_RES (34)..(34): 4Hyp
AGRPGEVGPPGPPGPAGEKGSPGADGPAGAPGTPGPQG

SEQ ID NO: 63 - protein, 36 aa, human
  MOD_RES (3)..(3): 4Hyp
  MOD_RES (12)..(12): 4Hyp
  MOD_RES (18)..(18): 4Hyp
  MOD_RES (35)..(35): 4Hyp
GPPGESGREGAPGAEGSPGRDGSPGAKGDRGETGPA

SEQ ID NO: 64 - protein, 39 aa, human
  MOD_RES (1)..(1): 4Hyp
  MOD_RES (14)..(14): 4Hyp
  MOD_RES (26)..(26): 4Hyp
PPGADGQPGAKGEPGDAGAKGDAGPPGPAGPAGPPGPIG

SEQ ID NO: 65 - protein, 39 aa, human; identical to SEQ ID NO: 64
  MOD_RES (1)..(1): 4Hyp
  MOD_RES (14)..(14): 4Hyp
  MOD_RES (25)..(25): 4Hyp
  MOD_RES (26)..(26): 4Hyp

SEQ ID NO: 66 - protein, 40 aa, human
  MOD_RES (3)..(3): 4Hyp
  MOD_RES (29)..(29): 4Hyp
  MOD_RES (36)..(36): 4Hyp
GPPGADGQPGAKGEPGDAGAKGDAGPPGPAGPAGPPGPIG

SEQ ID NO: 67 - protein, 40 aa, human; identical to SEQ ID NO: 66
  MOD_RES (3)..(3): 4Hyp
  MOD_RES (15)..(15): 4Hyp
  MOD_RES (29)..(29): 4Hyp
  MOD_RES (38)..(38): 4Hyp

SEQ ID NO: 68 - protein, 40 aa, human
  MOD_RES (14)..(14): 4Hyp
GSEGPQGVRGEPGPPGPAGAAGPAGNPGADGQPGAKGANG

SEQ ID NO: 69 - protein, 37 aa, human
  MOD_RES (25)..(25): 4Hyp
  MOD_RES (26)..(26): 4Hyp
  MOD_RES (28)..(28): 4Hyp
  MOD_RES (29)..(29): 4Hyp
DKGETGEQGDRGIKGHRGFSGLQGPPGPPGSPGEQGP

SEQ ID NO: 70 - protein, 43 aa, human
  MOD_RES (9)..(9): 4Hyp
  MOD_RES (11)..(11): 4Hyp
  MOD_RES (14)..(14): 4Hyp
GERGVQGPPGPAGPRGANGAPGNDGAKGDAGAPGAPGSQGAPG

SEQ ID NO: 71 - protein, 42 aa, human
  MOD_RES (14)..(14): 4Hyp
  MOD_RES (16)..(16): 4Hyp
PAGKDGEAGAQGPPGPAGPAGERGEQGPAGSPGFQGLPGPAG